European Patent Specification EP 3 445 786 B1, published October 4, 2023. Title: Use of an agent capable of binding to CLEVER-1 in immune activation and methods based thereon. Applicant: Faron Pharmaceuticals Oy. The sequence listing filed with the application follows.

SEQUENCE LISTING (7 sequences)

SEQ ID NO: 1 - protein, 15 aa, Homo sapiens
PFTVLVPSVSSFSSR

SEQ ID NO: 2 - protein, 12 aa, Homo sapiens
QEITVTFNQFTK

SEQ ID NO: 3 - protein, 10 aa, Homo sapiens
ATQTGRVFLQ

SEQ ID NO: 4 - protein, 12 aa, Homo sapiens
DSLRDGRLIYLF

SEQ ID NO: 5 - protein, 13 aa, Homo sapiens
SKGRILTMANQVL

SEQ ID NO: 6 - protein, 15 aa, Homo sapiens
LCVYQKPGQAFCTCR

SEQ ID NO: 7 - protein, 1051 aa, Homo sapiens
LCCACLLELIPYAPTLSWTACPPAMAGPRGLLPLCLLAFCLAGFSFVRGQVLFKGCDVKTTFVTHVPCTSCAAIKKQTCPSGWLRELPDQITQDCRYEVQLGGSMVSMSGCRRKCRKQVVQKACCPGYWGSRCHECPGGAETPCNGHGTCLDGMDRNGTCVCQENFRGSACQECQDPNRFGPDCQSVCSCVHGVCNHGPRGDGSCLCFAGYTGPHCDQELPVCQELRCPQNTQCSAEAPSCRCLPGYTQQGSECRAPNPCWPSPCSLLAQCSVSPKGQAQCHCPENYHGDGMVCLPKDPCTDNLGGCPSNSTLCVYQKPGQAFCTCRPGLVSINSNASAGCFAFCSPFSCDRSATCQVTADGKTSCVCRESEVGDGRACYGHLLHEVQKATQTGRVFLQLRVAVAMMDQGCREILTTAGPFTVLVPSVSSFSSRTMNASLAQQLCRQHIIAGQHILEDTRTQQTRRWWTLAGQEITVTFNQFTKYSYKYKDQPQQTFNIYKANNIAANGVFHVVTGLRWQAPSGTPGDPKRTIGQILASTEAFSRFETILENCGLPSILDGPGPFTVFAPSNEAVDSLRDGRLIYLFTAGLSKLQELVRYHIYNHGQLTVEKLISKGRILTMANQVLAVNISEEGRILLGPEGVPLQRVDVMAANGVIHMLDGILLPPTILPILPKHCSEEQHKIVAGSCVDCQALNTSTCPPNSVKLDIFPKECVYIHDPTGLNVLKKGCASYCNQTIMEQGCCKGFFGPDCTQCPGGFSNPCYGKGNCSDGIQGNGACLCFPDYKGIACHICSNPNKHGEQCQEDCGCVHGLCDNRPGSGGVCQQGTCAPGFSGRFCNESMGDCGPTGLAQHCHLHARCVSQEGVARCRCLDGFEGDGFSCTPSNPCSHPDRGGCSENAECVPGSLGTHHCTCHKGWSGDGRVCVAIDECELDMRGGCHTDALCSYVGPGQSRCTCKLGFAGDGYQCSPIDPCRAGNGGCHGLATCRAVGGGQRVCTCPPGFGGDGFSCYGDIFRELEANAHFSIFYQWLKSAGITLPADRRVTALVPS